European Patent Application EP 4 345 173 A1, published April 3, 2024. Title: A method, uses, system and kit for detecting a human papillomavirus genotype associated with development of cervical, oral or anogenital cancer in a subject and for determining the genotype or genotypes thereof. Applicant: Vitro, S.A. Application EP. The sequence listing filed with the application follows.

SEQUENCE LISTING (56 sequences)

SEQ ID NO: 1 - DNA, 23 bp, synthetic construct
  source 1..23: mol_type = other DNA
tttgttactgtggtagatactac

SEQ ID NO: 2 - DNA, 25 bp, synthetic construct
  source 1..25: mol_type = other DNA
gaaaaataaactgtaaatcatattc

SEQ ID NO: 3 - DNA, 19 bp, synthetic construct
  source 1..19: mol_type = other DNA
gagccatctattgcttaca

SEQ ID NO: 4 - DNA, 18 bp, synthetic construct
  source 1..18: mol_type = other DNA
ctcaccaccaacttcatc

SEQ ID NO: 5 - DNA, 20 bp, synthetic construct
  source 1..20: mol_type = other DNA
gcagtacaaatatgtcatta

SEQ ID NO: 6 - DNA, 22 bp, synthetic construct
  source 1..22: mol_type = other DNA
caatatgatgctaccaaattta

SEQ ID NO: 7 - DNA, 21 bp, synthetic construct
  source 1..21: mol_type = other DNA
catttaaaagtagtaatttta

SEQ ID NO: 8 - DNA, 21 bp, synthetic construct
  source 1..21: mol_type = other DNA
cagtactaatatgactttatg

SEQ ID NO: 9 - DNA, 20 bp, synthetic construct
  source 1..20: mol_type = other DNA
ctagtgacagtacatataaa

SEQ ID NO: 10 - DNA, 21 bp, synthetic construct
  source 1..21: mol_type = other DNA
tagtaccaactttacattatc

SEQ ID NO: 11 - DNA, 23 bp, synthetic construct
  source 1..23: mol_type = other DNA
cagtactaatttaacattatgtg

SEQ ID NO: 12 - DNA, 22 bp, synthetic construct
  source 1..22: mol_type = other DNA
tacaaatttaactattagcact

SEQ ID NO: 13 - DNA, 23 bp, synthetic construct
  source 1..23: mol_type = other DNA
atataaaaatgaaaattttaagg

SEQ ID NO: 14 - DNA, 22 bp, synthetic construct
  source 1..22: mol_type = other DNA
agtactaacatgactattagta

SEQ ID NO: 15 - DNA, 24 bp, synthetic construct
  source 1..24: mol_type = other DNA
catataaaaatgataattttaagg

SEQ ID NO: 16 - DNA, 23 bp, synthetic construct
  source 1..23: mol_type = other DNA
cagcaccaatctttctgtgtgtg

SEQ ID NO: 17 - DNA, 23 bp, synthetic construct
  source 1..23: mol_type = other DNA
atatgatgcacgtgaaatcaatc

SEQ ID NO: 18 - DNA, 25 bp, synthetic construct
  source 1..25: mol_type = other DNA
tttatgattctaataaatttaagga

SEQ ID NO: 19 - DNA, 16 bp, synthetic construct
  source 1..16: mol_type = other DNA
tgcttctgacacaact

SEQ ID NO: 20 - DNA, 18 bp, synthetic construct
  source 1..18: mol_type = other DNA
gagtacctacgacatggg

SEQ ID NO: 21 - DNA, 20 bp, synthetic construct
  source 1..20: mol_type = other DNA
gcagtatagcagacatgttg

SEQ ID NO: 22 - DNA, 22 bp, synthetic construct
  source 1..22: mol_type = other DNA
agagtatttaagacatggtgag

SEQ ID NO: 23 - DNA, 25 bp, synthetic construct
  source 1..25: mol_type = other DNA
aaagaatatataagacatgttgaag

SEQ ID NO: 24 - DNA, 22 bp, synthetic construct
  source 1..22: mol_type = other DNA
ggaatatttaaggcatggtgaa

SEQ ID NO: 25 - DNA, 19 bp, synthetic construct
  source 1..19: mol_type = other DNA
ggaatataccaggcacgtg

SEQ ID NO: 26 - DNA, 22 bp, synthetic construct
  source 1..22: mol_type = other DNA
agtacatatgaccctactaagt

SEQ ID NO: 27 - DNA, 24 bp, synthetic construct
  source 1..24: mol_type = other DNA
tccaagtaactttaagcaatatat

SEQ ID NO: 28 - DNA, 19 bp, synthetic construct
  source 1..19: mol_type = other DNA
ggaataccttcgtcatggc

SEQ ID NO: 29 - DNA, 20 bp, synthetic construct
  source 1..20: mol_type = other DNA
tcagtaccttagacatgtgg

SEQ ID NO: 30 - DNA, 22 bp, synthetic construct
  source 1..22: mol_type = other DNA
ggaatatgtacgtcatgttgaa

SEQ ID NO: 31 - DNA, 20 bp, synthetic construct
  source 1..20: mol_type = other DNA
agaatatgccagacatgtgg

SEQ ID NO: 32 - DNA, 19 bp, synthetic construct
  source 1..19: mol_type = other DNA
tcaataccttcgccatgtg

SEQ ID NO: 33 - DNA, 22 bp, synthetic construct
  source 1..22: mol_type = other DNA
ggaatatattaggcatgttgag

SEQ ID NO: 34 - DNA, 24 bp, synthetic construct
  source 1..24: mol_type = other DNA
aaacaatttataagacatggcgaa

SEQ ID NO: 35 - DNA, 21 bp, synthetic construct
  source 1..21: mol_type = other DNA
aacagtatgttagacatgcag

SEQ ID NO: 36 - DNA, 24 bp, synthetic construct
  source 1..24: mol_type = other DNA
aaggaatatttaagacatgcagaa

SEQ ID NO: 37 - DNA, 19 bp, synthetic construct
  source 1..19: mol_type = other DNA
gcagtacattaggcatggg

SEQ ID NO: 38 - DNA, 21 bp, synthetic construct
  source 1..21: mol_type = other DNA
tataaagagtacatgcgtcat

SEQ ID NO: 39 - DNA, 18 bp, synthetic construct
  source 1..18: mol_type = other DNA
gaatacatgcgccatgtg

SEQ ID NO: 40 - DNA, 18 bp, synthetic construct
  source 1..18: mol_type = other DNA
ggaatatttgcgtcatgg

SEQ ID NO: 41 - DNA, 24 bp, synthetic construct
  source 1..24: mol_type = other DNA
ctaattttaaggaatatttaagac

SEQ ID NO: 42 - DNA, 20 bp, synthetic construct
  source 1..20: mol_type = other DNA
ttaaggaatacytgcggcat

SEQ ID NO: 43 - DNA, 20 bp, synthetic construct
  source 1..20: mol_type = other DNA
caatacatgcgacatgttga

SEQ ID NO: 44 - DNA, 20 bp, synthetic construct
  source 1..20: mol_type = other DNA
gagtatatwagacatgtgga

SEQ ID NO: 45 - DNA, 22 bp, synthetic construct
  source 1..22: mol_type = other DNA
aatataaacaatacatgcgaca

SEQ ID NO: 46 - DNA, 23 bp, synthetic construct
  source 1..23: mol_type = other DNA
ctttagggaatatttgcgccata

SEQ ID NO: 47 - DNA, 21 bp, synthetic construct
  source 1..21: mol_type = other DNA
aggcyaccaactttagggaat

SEQ ID NO: 48 - DNA, 20 bp, synthetic construct
  source 1..20: mol_type = other DNA
aataccttagacatgtggaa

SEQ ID NO: 49 - DNA, 22 bp, synthetic construct
  source 1..22: mol_type = other DNA
ttataagcagtttataaggcat

SEQ ID NO: 50 - DNA, 24 bp, synthetic construct
  source 1..24: mol_type = other DNA
tatatagccctacaaagtttaagg

SEQ ID NO: 51 - DNA, 20 bp, synthetic construct
  source 1..20: mol_type = other DNA
taaagcctctagtttcatgg

SEQ ID NO: 52 - DNA, 18 bp, synthetic construct
  source 1..18: mol_type = other DNA
tatcttcgccacactgag

SEQ ID NO: 53 - DNA, 19 bp, synthetic construct
  source 1..19: mol_type = other DNA
aatttctgcgccatacaga

SEQ ID NO: 54 - DNA, 19 bp, synthetic construct
  source 1..19: mol_type = other DNA
aatacctaagacatgtgga

SEQ ID NO: 55 - DNA, 14 bp, synthetic construct
  source 1..14: mol_type = other DNA
tgcttctgacacaa

SEQ ID NO: 56 - DNA, 16 bp, synthetic construct
  source 1..16: mol_type = other DNA
mgdcatgyygargaat